European Patent Application EP 4 223 779 A1, published August 9, 2023. Title: Chimeric Antigen Receptor Targeting EGFR. Applicant: INSTITUTE OF ZOOLOGY, CHINESE ACADEMY OF SCIENCES BEIJING INSTITUTE FOR STEM CELL AND REGENERATIVE MEDICINE. The sequence listing filed with the application follows.

SEQUENCE LISTING (82 sequences)

SEQ ID NO: 1 - protein, 6 aa, Artificial Sequence
  hu806 VH-CDR1
SDFAWN

SEQ ID NO: 2 - protein, 16 aa, Artificial Sequence
  hu806 VH-CDR2
YISYSGNTRYQPSLKS

SEQ ID NO: 3 - protein, 9 aa, Artificial Sequence
  hu806 VH-CDR3
VTAGRGFPY

SEQ ID NO: 4 - protein, 11 aa, Artificial Sequence
  hu806 VL-CDR1
HSSQDINSNIG

SEQ ID NO: 5 - protein, 7 aa, Artificial Sequence
  hu806 VL-CDR2
HGTNLDD

SEQ ID NO: 6 - protein, 9 aa, Artificial Sequence
  hu806 VL-CDR3
VQYAQFPWT

SEQ ID NO: 7 - protein, 116 aa, Artificial Sequence
  hu806 VH
QVQLQESGPGLVKPSQTLSLTCTVSGYSISSDFAWNWIRQPPGKGLEWMGYISYSGNTRYQPSLKSRITISRDTSKNQFFLKLNSVTAADTATYYCVTAGRGFPYWGQGTLVTVSS

SEQ ID NO: 8 - protein, 108 aa, Artificial Sequence
  hu806 VL
DIQMTQSPSSMSVSVGDRVTITCHSSQDINSNIGWLQQKPGKSFKGLIYHGTNLDDGVPSRFSGSGSGTDYTLTISSLQPEDFATYYCVQYAQFPWTFGGGTKLEIKR

SEQ ID NO: 9 - protein, 239 aa, Artificial Sequence
  hu806 ScFv
QVQLQESGPGLVKPSQTLSLTCTVSGYSISSDFAWNWIRQPPGKGLEWMGYISYSGNTRYQPSLKSRITISRDTSKNQFFLKLNSVTAADTATYYCVTAGRGFPYWGQGTLVTVSSGGGGSGGGGSGGGGSDIQMTQSPSSMSVSVGDRVTITCHSSQDINSNIGWLQQKPGKSFKGLIYHGTNLDDGVPSRFSGSGSGTDYTLTISSLQPEDFATYYCVQYAQFPWTFGGGTKLEIKR

SEQ ID NO: 10 - protein, 4 aa, Artificial Sequence
  E2 VH-CDR1
NYDM

SEQ ID NO: 11 - protein, 17 aa, Artificial Sequence
  E2 VH-CDR2
GISHSSGSKYYADSVKG

SEQ ID NO: 12 - protein, 13 aa, Artificial Sequence
  E2 VH-CDR3
KDATPRPLKPFDY

SEQ ID NO: 13 - protein, 13 aa, Artificial Sequence
  E2 VL-CDR1
TGSSSNIGNNDVS

SEQ ID NO: 14 - protein, 7 aa, Artificial Sequence
  E2 VL-CDR2
DDNKRPS

SEQ ID NO: 15 - protein, 9 aa, Artificial Sequence
  E2 VL-CDR3
GSWDASLNA

SEQ ID NO: 16 - protein, 121 aa, Artificial Sequence
  E2 VH
EVQLLESGGGLVQPGGSLRLSCAASGFTFSNYDMSWVRQAPGKGLEWVSGISHSSGSKYYADSVKGRFTISRDNSKNTLYLQMNSLRAEDTAVYYCAKDATPRPLKPFDYWGQGTLVTVSS

SEQ ID NO: 17 - protein, 111 aa, Artificial Sequence
  E2 VL
QSVLTQPPSASGTPGQRVTISCTGSSSNIGNNDVSWYQQLPGTAPKLLIYDDNKRPSGVPDRFSGSKSGTSASLAISGLRSEDEADYYCGSWDASLNAYVFGGGTKLTVLG

SEQ ID NO: 18 - protein, 247 aa, Artificial Sequence
  E2 ScFv
EVQLLESGGGLVQPGGSLRLSCAASGFTFSNYDMSWVRQAPGKGLEWVSGISHSSGSKYYADSVKGRFTISRDNSKNTLYLQMNSLRAEDTAVYYCAKDATPRPLKPFDYWGQGTLVTVSSGGGGSGGGGSGGGGSQSVLTQPPSASGTPGQRVTISCTGSSSNIGNNDVSWYQQLPGTAPKLLIYDDNKRPSGVPDRFSGSKSGTSASLAISGLRSEDEADYYCGSWDASLNAYVFGGGTKLTVLG

SEQ ID NO: 19 - protein, 7 aa, Artificial Sequence
  Pan VH-CDR1
SGDYYWT

SEQ ID NO: 20 - protein, 16 aa, Artificial Sequence
  Pan VH-CDR2
HIYYSGNTNYNPSLKS

SEQ ID NO: 21 - protein, 9 aa, Artificial Sequence
  Pan VH-CDR3
DRVTGAFDI

SEQ ID NO: 22 - protein, 11 aa, Artificial Sequence
  Pan VL-CDR1
QASQDISNYLN

SEQ ID NO: 23 - protein, 7 aa, Artificial Sequence
  Pan VL-CDR2
DASNLET

SEQ ID NO: 24 - protein, 9 aa, Artificial Sequence
  Pan VL-CDR3
QHFDHLPLA

SEQ ID NO: 25 - protein, 135 aa, Artificial Sequence
  Pan VH
QVQLQESGPGLVKPSETLSLTCTVSGGSVSSGDYYWTWIRQSPGKGLEWIGHIYYSGNTNYNPSLKSRLTISIDTSKTQFSLKLSSVTAADTAIYYCVRDRVTGAFDIWGQGTMVTVSSASTKGPSVFPLAPCSR

SEQ ID NO: 26 - protein, 107 aa, Artificial Sequence [sequence omitted]

SEQ ID NO: 27 - protein, 257 aa, Artificial Sequence
  Pan ScFv
QVQLQESGPGLVKPSETLSLTCTVSGGSVSSGDYYWTWIRQSPGKGLEWIGHIYYSGNTNYNPSLKSRLTISIDTSKTQFSLKLSSVTAADTAIYYCVRDRVTGAFDIWGQGTMVTVSSASTKGPSVFPLAPCSRGGGGSGGGGSGGGGSDIQMTQSPSSLSASVGDRVTITCQASQDISNYLNWYQQKPGKAPKLLIYDASNLETGVPSRFSGSGSGTDFTFTISSLQPEDIATYFCQHFDHLPLAFGGGTKVEIK

SEQ ID NO: 28 - protein, 7 aa, Artificial Sequence
  Nec VH-CDR1
SGDYYWS

SEQ ID NO: 29 - protein, 16 aa, Artificial Sequence
  Nec VH-CDR2
YIYYSGSTDYNPSLKS

SEQ ID NO: 30 - protein, 11 aa, Artificial Sequence
  Nec VH-CDR3
VSIFGVGTFDY

SEQ ID NO: 31 - protein, 11 aa, Artificial Sequence
  Nec VL-CDR1
RASQSVSSYLA

SEQ ID NO: 32 - protein, 7 aa, Artificial Sequence
  Nec VL-CDR2
DASNRAT

SEQ ID NO: 33 - protein, 9 aa, Artificial Sequence
  Nec VL-CDR3
HQYGSTPLT

SEQ ID NO: 34 - protein, 121 aa, Artificial Sequence [sequence omitted]

SEQ ID NO: 35 - protein, 107 aa, Artificial Sequence [sequence omitted]

SEQ ID NO: 36 - protein, 243 aa, Artificial Sequence
  Nec ScFv
QVQLQESGPGLVKPSQTLSLTCTVSGGSISSGDYYWSWIRQPPGKGLEWIGYIYYSGSTDYNPSLKSRVTMSVDTSKNQFSLKVNSVTAADTAVYYCARVSIFGVGTFDYWGQGTLVTVSSGGGGSGGGGSGGGGSEIVMTQSPATLSLSPGERATLSCRASQSVSSYLAWYQQKPGQAPRLLIYDASNRATGIPARFSGSGSGTDFTLTISSLEPEDFAVYYCHQYGSTPLTFGGGTKAEIK

SEQ ID NO: 37 - protein, 16 aa, Artificial Sequence
  Nimo VH-CDR1
RSSQNIVHSNGNTYLD

SEQ ID NO: 38 - protein, 7 aa, Artificial Sequence
  Nimo VH-CDR2
KVSNRFS

SEQ ID NO: 39 - protein, 9 aa, Artificial Sequence
  Nimo VH-CDR3
FQYSHVPWT

SEQ ID NO: 40 - protein, 5 aa, Artificial Sequence
  Nimo VL-CDR1
NYYIY

SEQ ID NO: 41 - protein, 18 aa, Artificial Sequence
  Nimo VL-CDR2
GGINPTSGGSNFNEKFKT

SEQ ID NO: 42 - protein, 14 aa, Artificial Sequence
  Nimo VL-CDR3
QGLWFDSDGRGFDF

SEQ ID NO: 43 - protein, 123 aa, Artificial Sequence
  Nimo VH
QVQLQQSGAEVKKPGSSVKVSCKASGYTFTNYYIYWVRQAPGQGLEWIGGINPTSGGSNFNEKFKTRVTITVDESTNTAYMELSSLRSEDTAFYFCARQGLWFDSDGRGFDFWGQGSTVTVSS

SEQ ID NO: 44 - protein, 114 aa, Artificial Sequence
  Nimo VL
DIQMTQSPSSLSASVGDRVTITCRSSQNIVHSNGNTYLDWYQQTPGKAPKLLIYKVSNRFSGVPSRFSGSGSGTDFTFTISSLQPEDIATYYCFQYSHVPWTFGQGTKLQITRE

SEQ ID NO: 45 - protein, 252 aa, Artificial Sequence
  Nimo ScFv
DIQMTQSPSSLSASVGDRVTITCRSSQNIVHSNGNTYLDWYQQTPGKAPKLLIYKVSNRFSGVPSRFSGSGSGTDFTFTISSLQPEDIATYYCFQYSHVPWTFGQGTKLQITREGGGGSGGGGSGGGGSQVQLQQSGAEVKKPGSSVKVSCKASGYTFTNYYIYWVRQAPGQGLEWIGGINPTSGGSNFNEKFKTRVTITVDESTNTAYMELSSLRSEDTAFYFCARQGLWFDSDGRGFDFWGQGSTVTVSS

SEQ ID NO: 46 - protein, 7 aa, Artificial Sequence
  301 VH CDR1
GTFSSYA

SEQ ID NO: 47 - protein, 8 aa, Artificial Sequence
  301 VH CDR2
IIPIFGTA

SEQ ID NO: 48 - protein, 8 aa, Artificial Sequence
  301 VH CDR3
ARTRLKHQ

SEQ ID NO: 49 - protein, 6 aa, Artificial Sequence
  301 VL CDR1
SLRSYY

SEQ ID NO: 50 - protein, 4 aa, Artificial Sequence
  301 VL CDR2
GKNN

SEQ ID NO: 51 - protein, 9 aa, Artificial Sequence
  301 VL CDR3
NSRDSSGPV

SEQ ID NO: 52 - protein, 115 aa, Artificial Sequence
  301 VH
QVQLVQSGAEVKKPGSSVKVSCKASGGTFSSYAISWVRQAPGQGLEWMGGIIPIFGTANYAQKFQGRVTITADESTSTAYMELSSLRSEDTAVYYCARTRLKHQWGQGTLVTVSS

SEQ ID NO: 53 - protein, 111 aa, Artificial Sequence
  301 VL
LSSELTQDPAVSVALGQTVRITCQGDSLRSYYASWYQQKPGQAPVLVIYGKNNRPSGIPDRFSGSSSGNTASLTITGAQAEDEADYYCNSRDSSGPVFGGGTKLTVLGAAA

SEQ ID NO: 54 - protein, 242 aa, Artificial Sequence
  301 ScFv
MAQVQLVQSGAEVKKPGSSVKVSCKASGGTFSSYAISWVRQAPGQGLEWMGGIIPIFGTANYAQKFQGRVTITADESTSTAYMELSSLRSEDTAVYYCARTRLKHQWGQGTLVTVSSGGGGSGGGGSGGSALSSELTQDPAVSVALGQTVRITCQGDSLRSYYASWYQQKPGQAPVLVIYGKNNRPSGIPDRFSGSSSGNTASLTITGAQAEDEADYYCNSRDSSGPVFGGGTKLTVLGAAA

SEQ ID NO: 55 - protein, 21 aa, Artificial Sequence
  CD8α signal peptide
MALPVTALLLPLALLLHAARP

SEQ ID NO: 56 - protein, 44 aa, Artificial Sequence
  CD8α hinge region
TTTPAPRPPTPAPTIASQPLSLRPEACRPAAGGAVHTRGLDFAC

SEQ ID NO: 57 - protein, 23 aa, Artificial Sequence
  CD8α transmembrane region
YIWAPLAGTCGVLLLSLVITLYC

SEQ ID NO: 58 - protein, 42 aa, Artificial Sequence
  4-1BB cytoplasmic domain
KRGRKKLLYIFKQPFMRPVQTTQEEDGCSCRFPEEEEGGCEL

SEQ ID NO: 59 - protein, 112 aa, Artificial Sequence
  CD3ζ
RVKFSRSADAPAYQQGQNQLYNELNLGRREEYDVLDKRRGRDPEMGGKPRRKNPQEGLYNELQKDKMAEAYSEIGMKGERRRGKGHDGLYQGLSTATKDTYDALHMQALPPR

SEQ ID NO: 60 - protein, 485 aa, Artificial Sequence
  hu806 CAR amino acid sequence
MALPVTALLLPLALLLHAARPQVQLQESGPGLVKPSQTLSLTCTVSGYSISSDFAWNWIRQPPGKGLEWMGYISYSGNTRYQPSLKSRITISRDTSKNQFFLKLNSVTAADTATYYCVTAGRGFPYWGQGTLVTVSSGGGGSGGGGSGGGGSDIQMTQSPSSMSVSVGDRVTITCHSSQDINSNIGWLQQKPGKSFKGLIYHGTNLDDGVPSRFSGSGSGTDYTLTISSLQPEDFATYYCVQYAQFPWTFGGGTKLEIKRTRTTTPAPRPPTPAPTIASQPLSLRPEACRPAAGGAVHTRGLDFACDIYIWAPLAGTCGVLLLSLVITLYCKRGRKKLLYIFKQPFMRPVQTTQEEDGCSCRFPEEEEGGCELRVKFSRSADAPAYQQGQNQLYNELNLGRREEYDVLDKRRGRDPEMGGKPRRKNPQEGLYNELQKDKMAEAYSEIGMKGERRRGKGHDGLYQGLSTATKDTYDALHMQALPPR

SEQ ID NO: 61 - protein, 493 aa, Artificial Sequence
  E2 CAR amino acid sequence
MALPVTALLLPLALLLHAARPEVQLLESGGGLVQPGGSLRLSCAASGFTFSNYDMSWVRQAPGKGLEWVSGISHSSGSKYYADSVKGRFTISRDNSKNTLYLQMNSLRAEDTAVYYCAKDATPRPLKPFDYWGQGTLVTVSSGGGGSGGGGSGGGGSQSVLTQPPSASGTPGQRVTISCTGSSSNIGNNDVSWYQQLPGTAPKLLIYDDNKRPSGVPDRFSGSKSGTSASLAISGLRSEDEADYYCGSWDASLNAYVFGGGTKLTVLGTRTTTPAPRPPTPAPTIASQPLSLRPEACRPAAGGAVHTRGLDFACDIYIWAPLAGTCGVLLLSLVITLYCKRGRKKLLYIFKQPFMRPVQTTQEEDGCSCRFPEEEEGGCELRVKFSRSADAPAYQQGQNQLYNELNLGRREEYDVLDKRRGRDPEMGGKPRRKNPQEGLYNELQKDKMAEAYSEIGMKGERRRGKGHDGLYQGLSTATKDTYDALHMQALPPR

SEQ ID NO: 62 - protein, 503 aa, Artificial Sequence
  Pan CAR amino acid sequence
MALPVTALLLPLALLLHAARPQVQLQESGPGLVKPSETLSLTCTVSGGSVSSGDYYWTWIRQSPGKGLEWIGHIYYSGNTNYNPSLKSRLTISIDTSKTQFSLKLSSVTAADTAIYYCVRDRVTGAFDIWGQGTMVTVSSASTKGPSVFPLAPCSRGGGGSGGGGSGGGGSDIQMTQSPSSLSASVGDRVTITCQASQDISNYLNWYQQKPGKAPKLLIYDASNLETGVPSRFSGSGSGTDFTFTISSLQPEDIATYFCQHFDHLPLAFGGGTKVEIKTRTTTPAPRPPTPAPTIASQPLSLRPEACRPAAGGAVHTRGLDFACDIYIWAPLAGTCGVLLLSLVITLYCKRGRKKLLYIFKQPFMRPVQTTQEEDGCSCRFPEEEEGGCELRVKFSRSADAPAYQQGQNQLYNELNLGRREEYDVLDKRRGRDPEMGGKPRRKNPQEGLYNELQKDKMAEAYSEIGMKGERRRGKGHDGLYQGLSTATKDTYDALHMQALPPR

SEQ ID NO: 63 - protein, 489 aa, Artificial Sequence
  Nec CAR amino acid sequence
MALPVTALLLPLALLLHAARPQVQLQESGPGLVKPSQTLSLTCTVSGGSISSGDYYWSWIRQPPGKGLEWIGYIYYSGSTDYNPSLKSRVTMSVDTSKNQFSLKVNSVTAADTAVYYCARVSIFGVGTFDYWGQGTLVTVSSGGGGSGGGGSGGGGSEIVMTQSPATLSLSPGERATLSCRASQSVSSYLAWYQQKPGQAPRLLIYDASNRATGIPARFSGSGSGTDFTLTISSLEPEDFAVYYCHQYGSTPLTFGGGTKAEIKTRTTTPAPRPPTPAPTIASQPLSLRPEACRPAAGGAVHTRGLDFACDIYIWAPLAGTCGVLLLSLVITLYCKRGRKKLLYIFKQPFMRPVQTTQEEDGCSCRFPEEEEGGCELRVKFSRSADAPAYQQGQNQLYNELNLGRREEYDVLDKRRGRDPEMGGKPRRKNPQEGLYNELQKDKMAEAYSEIGMKGERRRGKGHDGLYQGLSTATKDTYDALHMQALPPR

SEQ ID NO: 64 - protein, 498 aa, Artificial Sequence
  Nimo CAR amino acid sequence
MALPVTALLLPLALLLHAARPDIQMTQSPSSLSASVGDRVTITCRSSQNIVHSNGNTYLDWYQQTPGKAPKLLIYKVSNRFSGVPSRFSGSGSGTDFTFTISSLQPEDIATYYCFQYSHVPWTFGQGTKLQITREGGGGSGGGGSGGGGSQVQLQQSGAEVKKPGSSVKVSCKASGYTFTNYYIYWVRQAPGQGLEWIGGINPTSGGSNFNEKFKTRVTITVDESTNTAYMELSSLRSEDTAFYFCARQGLWFDSDGRGFDFWGQGSTVTVSSTRTTTPAPRPPTPAPTIASQPLSLRPEACRPAAGGAVHTRGLDFACDIYIWAPLAGTCGVLLLSLVITLYCKRGRKKLLYIFKQPFMRPVQTTQEEDGCSCRFPEEEEGGCELRVKFSRSADAPAYQQGQNQLYNELNLGRREEYDVLDKRRGRDPEMGGKPRRKNPQEGLYNELQKDKMAEAYSEIGMKGERRRGKGHDGLYQGLSTATKDTYDALHMQALPPR

SEQ ID NO: 65 - protein, 488 aa, Artificial Sequence
  301 CAR amino acid sequence
MALPVTALLLPLALLLHAARPMAQVQLVQSGAEVKKPGSSVKVSCKASGGTFSSYAISWVRQAPGQGLEWMGGIIPIFGTANYAQKFQGRVTITADESTSTAYMELSSLRSEDTAVYYCARTRLKHQWGQGTLVTVSSGGGGSGGGGSGGSALSSELTQDPAVSVALGQTVRITCQGDSLRSYYASWYQQKPGQAPVLVIYGKNNRPSGIPDRFSGSSSGNTASLTITGAQAEDEADYYCNSRDSSGPVFGGGTKLTVLGAAATRTTTPAPRPPTPAPTIASQPLSLRPEACRPAAGGAVHTRGLDFACDIYIWAPLAGTCGVLLLSLVITLYCKRGRKKLLYIFKQPFMRPVQTTQEEDGCSCRFPEEEEGGCELRVKFSRSADAPAYQQGQNQLYNELNLGRREEYDVLDKRRGRDPEMGGKPRRKNPQEGLYNELQKDKMAEAYSEIGMKGERRRGKGHDGLYQGLSTATKDTYDALHMQALPPR

SEQ ID NO: 66 - DNA, 1458 bp, Artificial Sequence
  hu806 CAR nucleotide sequence
atggccttaccagtgaccgccttgctcctgccgctggccttgctgctccacgccgccaggccgcaggtgcagctccaagagagtggacctgggcttgtcaagccgagtcaaactttgtccctaacatgtactgtgtccggatactctatctcatcagattttgcgtggaattggataaggcagccaccagggaaaggtttagaatggatgggctacatatcatactctgggaacaccagatatcaaccttctctgaaaagccggatcacaatctcaagggacacgtcgaagaatcagttcttcctgaaactgaactccgttacagccgcagacacagcaacatattactgcgtaaccgctggcagaggcttcccctattggggacagggcaccctagtgacagtgagcagcggtggcggtggctcgggcggtggtgggtcgggtggcggcggatctgatattcagatgactcagagtccatccagcatgtcagtctccgtgggagatagggtgacgataacctgtcattcaagccaagacatcaactccaatattggatggctccaacagaagcctggtaagtccttcaaaggactaatctatcacggaacaaacttggacgacggcgtgccatcgagattttcagggtctggcagcgggaccgactatacactgaccatctctagcttacaaccagaggactttgccacatactactgcgtccagtacgctcagttcccctggacattcggcggcggcacaaaactggaaatcaaacgtacgcgtaccacgacgccagcgccgcgaccaccaacaccggcgcccaccatcgcgtcgcagcccctgtccctgcgcccagaggcgtgccggccagcggcggggggcgcagtgcacacgagggggctggacttcgcctgtgatatctacatctgggcgcccttggccgggacttgtggggtccttctcctgtcactggttatcaccctttactgcaaacggggcagaaagaaactcctgtatatattcaaacaaccatttatgagaccagtacaaactactcaagaggaagatggctgtagctgccgatttccagaagaagaagaaggaggatgtgaactgagagtgaagttcagcaggagcgcagacgcccccgcgtaccagcagggccagaaccagctctataacgagctcaatctaggacgaagagaggagtacgatgttttggacaagagacgtggccgggaccctgagatggggggaaagccgagaaggaagaaccctcaggaaggcctgtacaatgaactgcagaaagataagatggcggaggcctacagtgagattgggatgaaaggcgagcgccggaggggcaaggggcacgatggcctttaccagggtctcagtacagccaccaaggacacctacgacgcccttcacatgcaggccctgccccctcgctaa

SEQ ID NO: 67 - DNA, 1482 bp, Artificial Sequence
  E2 CAR
atggccttaccagtgaccgccttgctcctgccgctggccttgctgctccacgccgccaggccggaggtgcagctgttggagtctgggggaggcttggtacagcctggggggtccctgagactctcctgtgcagcctctggattcacctttagcaattatgatatgagctgggtccgccaggctccagggaaggggctggagtgggtctcagggatctctcatagtagtggtagtaaatattacgctgattctgtaaaaggtcggttcaccatctccagagacaattccaagaacacgctgtatctgcaaatgaacagcctgagagccgaggacacggccgtgtattactgtgcgaaagatgctactccgcgtccgctgaagcctttcgactactggggccagggtacactggtcaccgtgagctcaggtggcggtggctcgggcggtggtgggtcgggtggcggcggatctcagtctgtgctgactcagccaccctcagcgtctgggacccccgggcagagggtcaccatctcttgtactggctcttcatctaatattggcaataatgatgtctcctggtaccagcagctcccaggaacggcccccaaactcctcatctatgatgataataagcggccaagcggggtccctgaccgattctctggctccaaatctggcacctcagcctccctggccatcagtgggctccggtccgaggatgaggctgattattactgtggttcttgggatgctagcctgaatgcttatgtcttcggcggaggcaccaagctgacggtcctaggcacgcgtaccacgacgccagcgccgcgaccaccaacaccggcgcccaccatcgcgtcgcagcccctgtccctgcgcccagaggcgtgccggccagcggcggggggcgcagtgcacacgagggggctggacttcgcctgtgatatctacatctgggcgcccttggccgggacttgtggggtccttctcctgtcactggttatcaccctttactgcaaacggggcagaaagaaactcctgtatatattcaaacaaccatttatgagaccagtacaaactactcaagaggaagatggctgtagctgccgatttccagaagaagaagaaggaggatgtgaactgagagtgaagttcagcaggagcgcagacgcccccgcgtaccagcagggccagaaccagctctataacgagctcaatctaggacgaagagaggagtacgatgttttggacaagagacgtggccgggaccctgagatggggggaaagccgagaaggaagaaccctcaggaaggcctgtacaatgaactgcagaaagataagatggcggaggcctacagtgagattgggatgaaaggcgagcgccggaggggcaaggggcacgatggcctttaccagggtctcagtacagccaccaaggacacctacgacgcccttcacatgcaggccctgccccctcgctaa

SEQ ID NO: 68 - DNA, 1512 bp, Artificial Sequence
  Pan CAR
atggccttaccagtgaccgccttgctcctgccgctggccttgctgctccacgccgccaggccgcaggtgcaacttcaagagagcggccctggacttgtgaaacccagcgaaaccctgagcctgacatgtaccgtgagcggaggaagcgtgagcagcggagactactactggacctggatcagacagagccccggaaaaggccttgaatggatcggccacatctactacagcggcaacaccaactacaaccccagcctgaagagcagactgaccatcagcatcgacaccagcaagacccagttcagcctgaagctgagcagcgtgacagctgctgacaccgctatctactactgcgtgagagacagagtgaccggcgctttcgatatttggggccagggaacaatggtgaccgtgagcagcgctagcacaaaaggccctagcgtgtttcctcttgccccctgtagcagaggtggcggtggctcgggcggtggtgggtcgggtggcggcggatctgacatccagatgacacagagccctagcagcctgtctgctagcgttggagacagagtgaccatcacctgtcaagccagccaggacatcagcaactacctgaactggtaccagcagaaacctggcaaggctcccaaactgctgatttacgacgccagcaatctggaaacaggcgtgcctagcagatttagcggcagcggaagcggaaccgatttcaccttcaccatcagcagcctgcagcccgaagacattgccacctacttctgccagcacttcgatcatctgcccctggcctttggaggaggaacaaaggtggagatcaagacgcgtaccacgacgccagcgccgcgaccaccaacaccggcgcccaccatcgcgtcgcagcccctgtccctgcgcccagaggcgtgccggccagcggcggggggcgcagtgcacacgagggggctggacttcgcctgtgatatctacatctgggcgcccttggccgggacttgtggggtccttctcctgtcactggttatcaccctttactgcaaacggggcagaaagaaactcctgtatatattcaaacaaccatttatgagaccagtacaaactactcaagaggaagatggctgtagctgccgatttccagaagaagaagaaggaggatgtgaactgagagtgaagttcagcaggagcgcagacgcccccgcgtaccagcagggccagaaccagctctataacgagctcaatctaggacgaagagaggagtacgatgttttggacaagagacgtggccgggaccctgagatggggggaaagccgagaaggaagaaccctcaggaaggcctgtacaatgaactgcagaaagataagatggcggaggcctacagtgagattgggatgaaaggcgagcgccggaggggcaaggggcacgatggcctttaccagggtctcagtacagccaccaaggacacctacgacgcccttcacatgcaggccctgccccctcgctaa

SEQ ID NO: 69 - DNA, 1470 bp, Artificial Sequence
  Nec CAR
atggccttaccagtgaccgccttgctcctgccgctggccttgctgctccacgccgccaggccgcaggtgcagctgcaggagtcgggcccaggactggtgaagccttcacagaccctgtccctcacctgcactgtctctggtggctccatcagcagtggtgattactactggagttggatccgccagcccccagggaagggcctggagtggattgggtacatctattacagtgggagcaccgactacaacccgtccctcaagagtcgagtcaccatgtccgtagacacgtccaagaatcagttttccctgaaggtcaactctgtgaccgccgcagacacggctgtgtattactgtgcgagagtgtcgatttttggagtggggacatttgactactggggccagggcaccctggtcaccgtctcaagcggtggcggtggctcgggcggtggtgggtcgggtggcggcggatctgaaattgtgatgacacagtctccagccaccctgtctttgtctccaggggaaagagccaccctctcctgcagggccagtcagagtgttagcagctacttagcctggtaccaacagaaacctggccaggctcccaggctcctcatctatgatgcatccaacagggccactggcatcccagccaggttcagtggcagtgggtctgggacagacttcactctcaccatcagcagcctagagcctgaagattttgcagtgtattactgtcaccagtatggtagcacacctctcactttcggcggagggaccaaggcggagatcaaaacgcgtaccacgacgccagcgccgcgaccaccaacaccggcgcccaccatcgcgtcgcagcccctgtccctgcgcccagaggcgtgccggccagcggcggggggcgcagtgcacacgagggggctggacttcgcctgtgatatctacatctgggcgcccttggccgggacttgtggggtccttctcctgtcactggttatcaccctttactgcaaacggggcagaaagaaactcctgtatatattcaaacaaccatttatgagaccagtacaaactactcaagaggaagatggctgtagctgccgatttccagaagaagaagaaggaggatgtgaactgagagtgaagttcagcaggagcgcagacgcccccgcgtaccagcagggccagaaccagctctataacgagctcaatctaggacgaagagaggagtacgatgttttggacaagagacgtggccgggaccctgagatggggggaaagccgagaaggaagaaccctcaggaaggcctgtacaatgaactgcagaaagataagatggcggaggcctacagtgagattgggatgaaaggcgagcgccggaggggcaaggggcacgatggcctttaccagggtctcagtacagccaccaaggacacctacgacgcccttcacatgcaggccctgccccctcgctaa

SEQ ID NO: 70 - DNA, 1497 bp, Artificial Sequence
  Nimo CAR
atggccttaccagtgaccgccttgctcctgccgctggccttgctgctccacgccgccaggccggacatccagatgacccagagcccaagcagcctgagcgccagcgtgggtgacagagtgaccatcacctgtagatctagtcagaacattgtacatagtaatggaaacacctatttagactggtaccagcagacgccaggtaaggctccaaagctgctgatctacaaagtttccaaccgatttagcggtgtgccaagcagattcagcggtagcggtagcggtaccgacttcaccttcaccatcagcagcctccagccagaggacatcgccacctactactgctttcaatactcacatgttccgtggacgtttggtcagggtactaagcttcaaatcactagggaaggtggcggtggctcgggcggtggtgggtcgggtggcggcggatctcaggtccaactgcagcagtctggggctgaagtgaagaagcctgggtcatcagtgaaggtgtcctgcaaggcttctggctacaccttcaccaactactatatttactgggtgcgacaggcccctggacaagggcttgagtggattggagggattaatcctactagcggtggtagcaacttcaatgagaagttcaagactagagtgaccatcaccgtggacgaatccacgaacacagcctacatggagctgagcagcctgagatctgaggacacggccttctatttctgtgcgagacaagggctttggtttgatagcgatgggcgaggttttgatttctggggccaagggtctacggtcaccgtctcctcaacgcgtaccacgacgccagcgccgcgaccaccaacaccggcgcccaccatcgcgtcgcagcccctgtccctgcgcccagaggcgtgccggccagcggcggggggcgcagtgcacacgagggggctggacttcgcctgtgatatctacatctgggcgcccttggccgggacttgtggggtccttctcctgtcactggttatcaccctttactgcaaacggggcagaaagaaactcctgtatatattcaaacaaccatttatgagaccagtacaaactactcaagaggaagatggctgtagctgccgatttccagaagaagaagaaggaggatgtgaactgagagtgaagttcagcaggagcgcagacgcccccgcgtaccagcagggccagaaccagctctataacgagctcaatctaggacgaagagaggagtacgatgttttggacaagagacgtggccgggaccctgagatggggggaaagccgagaaggaagaaccctcaggaaggcctgtacaatgaactgcagaaagataagatggcggaggcctacagtgagattgggatgaaaggcgagcgccggaggggcaaggggcacgatggcctttaccagggtctcagtacagccaccaaggacacctacgacgcccttcacatgcaggccctgccccctcgctaa

SEQ ID NO: 71 - DNA, 1467 bp, Artificial Sequence
  301 CAR
atggccttaccagtgaccgccttgctcctgccgctggccttgctgctccacgccgccaggccgatggcccaggtgcagctggtgcagtctggggctgaggtgaagaagcctgggtcctcggtgaaggtctcctgcaaggcttctggaggcaccttcagcagctatgctatcagctgggtgcgacaggcccctggacaagggcttgagtggatgggagggatcatccctatctttggtacagcaaactacgcacagaagttccagggcagagtcacgattaccgcggacgaatccacgagcacagcctacatggagctgagcagcctgagatctgaggacacggccgtgtattactgtgcaagaactcggcttaagcatcagtggggccaaggtaccctggtcaccgtctcgagtggtggaggcggttcaggcggaggtggctctggcggtagtgcactttcttctgagctgactcaggaccctgctgtgtctgtggccttgggacagacagtcaggatcacatgccaaggagacagcctcagaagctattatgcaagctggtaccagcagaagccaggacaggcccctgtacttgtcatctatggtaaaaacaaccggccctcagggatcccagaccgattctctggctccagctcaggaaacacagcttccttgaccatcactggggctcaggcggaagatgaggctgactattactgtaactcccgggacagcagtggtccggtattcggcggagggaccaagctgaccgtcctaggtgcggccgcaacgcgtaccacgacgccagcgccgcgaccaccaacaccggcgcccaccatcgcgtcgcagcccctgtccctgcgcccagaggcgtgccggccagcggcggggggcgcagtgcacacgagggggctggacttcgcctgtgatatctacatctgggcgcccttggccgggacttgtggggtccttctcctgtcactggttatcaccctttactgcaaacggggcagaaagaaactcctgtatatattcaaacaaccatttatgagaccagtacaaactactcaagaggaagatggctgtagctgccgatttccagaagaagaagaaggaggatgtgaactgagagtgaagttcagcaggagcgcagacgcccccgcgtaccagcagggccagaaccagctctataacgagctcaatctaggacgaagagaggagtacgatgttttggacaagagacgtggccgggaccctgagatggggggaaagccgagaaggaagaaccctcaggaaggcctgtacaatgaactgcagaaagataagatggcggaggcctacagtgagattgggatgaaaggcgagcgccggaggggcaaggggcacgatggcctttaccagggtctcagtacagccaccaaggacacctacgacgcccttcacatgcaggccctgccccctcgctaa

SEQ ID NO: 72 - protein, 15 aa, Artificial Sequence
  peptide linker
GGGGSGGGGSGGGGS

SEQ ID NO: 73 - protein, 239 aa, Artificial Sequence
  m806 ScFv
DVQLQESGPSLVKPSQSLSLTCTVTGYSITSDFAWNWIRQFPGNKLEWMGYISYSGNTRYNPSLKSRISITRDTSKNQFFLQLNSVTIEDTATYYCVTAGRGFPYWGQGTLVTVSAGGGGSGGGGSGGGGSDILMTQSPSSMSVSLGDTVSITCHSSQDINSNIGWLQQRPGKSFKGLIYHGTNLDDEVPSRFSGSGSGADYSLTISSLESEDFADYYCVQYAQFPWTFGGGTKLEIKR

SEQ ID NO: 74 - DNA, 717 bp, Artificial Sequence
  m806 ScFv
gatgtgcagcttcaggagtcgggacctagcctggtgaaaccttctcagtctctgtccctcacctgcactgtcactggctactcaatcaccagtgattttgcctggaactggatccggcagtttccaggaaacaagctggagtggatgggctacataagttatagtggtaacactaggtacaacccatctctcaaaagtcgaatctctatcactcgagacacatccaagaaccaattcttcctgcagttgaattctgtgactattgaggacacagccacatattactgtgtaacggcgggacgcgggtttccttattggggccaagggactctggtcactgtctctgcaggtggcggtggctcgggcggtggtgggtcgggtggcggcggatctgacatcctgatgacccaatctccatcctccatgtctgtatctctgggagacacagtcagcatcacttgccattcaagtcaggacattaacagtaatatagggtggttgcagcagagaccagggaaatcatttaagggcctgatctatcatggaaccaacttggacgatgaagttccatcaaggttcagtggcagtggatctggagccgattattctctcaccatcagcagcctggaatctgaagattttgcagactattactgtgtacagtatgctcagtttccgtggacgttcggtggaggcaccaagctggaaatcaaacgt

SEQ ID NO: 75 - protein, 6 aa, Artificial Sequence
  m806 ScFv VH CDR1
SDFAWN

SEQ ID NO: 76 - protein, 16 aa, Artificial Sequence
  m806 ScFv VH CDR2
YISYSGNTRYNPSLKS

SEQ ID NO: 77 - protein, 9 aa, Artificial Sequence
  m806 ScFv VH CDR3
VTAGRGFPY

SEQ ID NO: 78 - protein, 11 aa, Artificial Sequence
  m806 ScFv VL CDR1
HSSQDINSNIG

SEQ ID NO: 79 - protein, 7 aa, Artificial Sequence
  m806 ScFv VL CDR2
HGTNLDD

SEQ ID NO: 80 - protein, 9 aa, Artificial Sequence
  m806 ScFv VL CDR3
VQYAQFPWT

SEQ ID NO: 81 - protein, 485 aa, Artificial Sequence
  m806 CAR
MALPVTALLLPLALLLHAARPDVQLQESGPSLVKPSQSLSLTCTVTGYSITSDFAWNWIRQFPGNKLEWMGYISYSGNTRYNPSLKSRISITRDTSKNQFFLQLNSVTIEDTATYYCVTAGRGFPYWGQGTLVTVSAGGGGSGGGGSGGGGSDILMTQSPSSMSVSLGDTVSITCHSSQDINSNIGWLQQRPGKSFKGLIYHGTNLDDEVPSRFSGSGSGADYSLTISSLESEDFADYYCVQYAQFPWTFGGGTKLEIKRTRTTTPAPRPPTPAPTIASQPLSLRPEACRPAAGGAVHTRGLDFACDIYIWAPLAGTCGVLLLSLVITLYCKRGRKKLLYIFKQPFMRPVQTTQEEDGCSCRFPEEEEGGCELRVKFSRSADAPAYQQGQNQLYNELNLGRREEYDVLDKRRGRDPEMGGKPRRKNPQEGLYNELQKDKMAEAYSEIGMKGERRRGKGHDGLYQGLSTATKDTYDALHMQALPPR

SEQ ID NO: 82 - DNA, 1470 bp, Artificial Sequence
  m806 CAR
ggatccatggccttaccagtgaccgccttgctcctgccgctggccttgctgctccacgccgccaggccggatgtgcagcttcaggagtcgggacctagcctggtgaaaccttctcagtctctgtccctcacctgcactgtcactggctactcaatcaccagtgattttgcctggaactggatccggcagtttccaggaaacaagctggagtggatgggctacataagttatagtggtaacactaggtacaacccatctctcaaaagtcgaatctctatcactcgagacacatccaagaaccaattcttcctgcagttgaattctgtgactattgaggacacagccacatattactgtgtaacggcgggacgcgggtttccttattggggccaagggactctggtcactgtctctgcaggtggcggtggctcgggcggtggtgggtcgggtggcggcggatctgacatcctgatgacccaatctccatcctccatgtctgtatctctgggagacacagtcagcatcacttgccattcaagtcaggacattaacagtaatatagggtggttgcagcagagaccagggaaatcatttaagggcctgatctatcatggaaccaacttggacgatgaagttccatcaaggttcagtggcagtggatctggagccgattattctctcaccatcagcagcctggaatctgaagattttgcagactattactgtgtacagtatgctcagtttccgtggacgttcggtggaggcaccaagctggaaatcaaacgtacgcgtaccacgacgccagcgccgcgaccaccaacaccggcgcccaccatcgcgtcgcagcccctgtccctgcgcccagaggcgtgccggccagcggcggggggcgcagtgcacacgagggggctggacttcgcctgtgatatctacatctgggcgcccttggccgggacttgtggggtccttctcctgtcactggttatcaccctttactgcaaacggggcagaaagaaactcctgtatatattcaaacaaccatttatgagaccagtacaaactactcaagaggaagatggctgtagctgccgatttccagaagaagaagaaggaggatgtgaactgagagtgaagttcagcaggagcgcagacgcccccgcgtaccagcagggccagaaccagctctataacgagctcaatctaggacgaagagaggagtacgatgttttggacaagagacgtggccgggaccctgagatggggggaaagccgagaaggaagaaccctcaggaaggcctgtacaatgaactgcagaaagataagatggcggaggcctacagtgagattgggatgaaaggcgagcgccggaggggcaaggggcacgatggcctttaccagggtctcagtacagccaccaaggacacctacgacgcccttcacatgcaggccctgccccctcgctaagtcgac